European Patent Application EP 4 269 598 A1, published November 1, 2023. Title: A microorganism of the genus Corynebacterium producing L-amino acids and method for producing L-amino acids using the same. Applicant: CJ CheilJedang Corporation. The sequence listing filed with the application follows.

SEQUENCE LISTING (48 sequences)

SEQ ID NO: 1 - protein, 484 aa, Artificial Sequence
  zwf (C.gl 13032)
MVIFGVTGDLARKKLLPAIYDLANRGLLPPGFSLVGYGRREWSKEDFEKYVRDAASAGARTEFRENVWERLAEGMEFVRGNFDDDAAFDNLAATLKRIDKTRGTAGNWAYYLSIPPDSFTAVCHQLERSGMAESTEEAWRRVIIEKPFGHNLESAHELNQLVNAVFPESSVFRIDHYLGKETVQNILALRFANQLFEPLWNSNYVDHVQITMAEDIGLGGRAGYYDGIGAARDVIQNHLIQLLALVAMEEPISFVPAQLQAEKIKVLSATKPCYPLDKTSARGQYAAGWQGSELVKGLREEDGFNPESTTETFAACTLEITSRRWAGVPFYLRTGKRLGRRVTEIAVVFKDAPHQPFDGDMTVSLGQNAIVIRVQPDEGVLIRFGSKVPGSAMEVRDVNMDFSYSESFTEESPEAYERLILDALLDESSLFPTNEEVELSWKILDPILEAWDADGEPEDYPAGTWGPKSADEMLSRNGHTWRRP

SEQ ID NO: 2 - DNA, 1545 bp, Artificial Sequence
  zwf (C.gl 13032)
gtgagcacaaacacgaccccctccagctggacaaacccactgcgcgacccgcaggataaacgactcccccgcatcgctggcccttccggcatggtgatcttcggtgtcactggcgacttggctcgaaagaagctgctccccgccatttatgatctagcaaaccgcggattgctgcccccaggattctcgttggtaggttacggccgccgcgaatggtccaaagaagactttgaaaaatacgtacgcgatgccgcaagtgctggtgctcgtacggaattccgtgaaaatgtttgggagcgcctcgccgagggtatggaatttgttcgcggcaactttgatgatgatgcagctttcgacaacctcgctgcaacactcaagcgcatcgacaaaacccgcggcaccgccggcaactgggcttactacctgtccattccaccagattccttcacagcggtctgccaccagctggagcgttccggcatggctgaatccaccgaagaagcatggcgccgcgtgatcatcgagaagcctttcggccacaacctcgaatccgcacacgagctcaaccagctggtcaacgcagtcttcccagaatcttctgtgttccgcatcgaccactatttgggcaaggaaacagttcaaaacatcctggctctgcgttttgctaaccagctgtttgagccactgtggaactccaactacgttgaccacgtccagatcaccatggctgaagatattggcttgggtggacgtgctggttactacgacggcatcggcgcagcccgcgacgtcatccagaaccacctgatccagctcttggctctggttgccatggaagaaccaatttctttcgtgccagcgcagctgcaggcagaaaagatcaaggtgctctctgcgacaaagccgtgctacccattggataaaacctccgctcgtggtcagtacgctgccggttggcagggctctgagttagtcaagggacttcgcgaagaagatggcttcaaccctgagtccaccactgagacttttgcggcttgtaccttagagatcacgtctcgtcgctgggctggtgtgccgttctacctgcgcaccggtaagcgtcttggtcgccgtgttactgagattgccgtggtgtttaaagacgcaccacaccagcctttcgacggcgacatgactgtatcccttggccaaaacgccatcgtgattcgcgtgcagcctgatgaaggtgtgctcatccgcttcggttccaaggttccaggttctgccatggaagtccgtgacgtcaacatggacttctcctactcagaatccttcactgaagaatcacctgaagcatacgagcgcctcattttggatgcgctgttagatgaatccagcctcttccctaccaacgaggaagtggaactgagctggaagattctggatccaattcttgaagcatgggatgccgatggagaaccagaggattacccagcgggtacgtggggtccaaagagcgctgatgaaatgctttcccgcaacggtcacacctggcgcaggccataa

SEQ ID NO: 3 - protein, 514 aa, Artificial Sequence
  zwf(C.gl 13869)
MSTNTTPTSWTNPLRDPQDKRLPRIAGPSGMVIFGVTGDLARKKLLPAIYDLANRGLLPPGFSLVGYGRREWSKEDFEKYVRDAASAGARTEFRENVWERLAEGMEFVRGNFDDDAAFDNLAATLKRIDKTRGTAGNWAYYLSIPPDSFTAVCHQLERSGMAESTEEAWRRVIIEKPFGHNLESAHELNQLVNAVFPESSVFRIDHYLGKETVQNILALRFANQLFEPLWNSNYVDHVQITMAEDIGLGGRAGYYDGIGAARDVIQNHLIQLLALVAMEEPISFVPAQLQAEKIKVLSATKPCYPLDKTSARGQYAAGWQGSELVKGLREEDGFNPESTTETFAACTLEITSRRWAGVPFYLRTGKRLGRRVTEIAVVFKDAPHQPFDGDMTVSLGQNAIVIRVQPDEGVLIRFGSKVPGSAMEVRDVNMDFSYSESFTEESPEAYERLILDALLDESSLFPTNEEVELSWKILDPILEAWDADGEPEDYPAGTWGPKSADEMLSRNGHTWRRP

SEQ ID NO: 4 - DNA, 1545 bp, Artificial Sequence
  zwf(C.gl 13869)
gtgagcacaaacacgacccccaccagctggacaaacccactgcgcgacccgcaggataaacgactcccccgcatcgctggcccttccggcatggtgatcttcggtgtcactggcgacttggctcgaaagaagctgcttcccgccatttatgatctagcaaaccgcggattgctgcccccaggattctcgttggtaggttacggccgccgcgaatggtccaaagaagactttgaaaaatacgtacgcgatgccgcaagtgctggtgctcgtacggaatttcgtgaaaatgtttgggagcgcctcgccgagggtatggaatttgttcgcggcaactttgatgatgatgcagctttcgacaacctcgctgcaacactcaagcgcatcgacaaaacccgcggcaccgccggcaactgggcttactacctgtccattccaccagattccttcacagcggtctgccaccagctggagcgttccggcatggctgaatccaccgaagaagcatggcgccgcgtgatcatcgagaagcctttcggccacaacctcgaatccgcacacgagctcaaccagctggtcaacgcagtcttcccagaatcttctgtgttccgcatcgaccactatttgggcaaggaaacagttcaaaacatcctggctctgcgttttgctaaccagctgtttgagccactgtggaactccaactacgttgaccacgtccagatcaccatggctgaagatatcggcttgggtggacgtgctggttactacgacggcatcggtgcagcccgcgacgtcatccagaaccacctgatccagctcttggctctggttgccatggaagaaccaatttctttcgtgccagcgcagctgcaggcagaaaagatcaaggtgctctctgcgacaaagccatgctacccattggataaaacctccgctcgtggtcagtacgctgccggttggcagggctctgagttagtcaagggacttcgcgaagaagatggcttcaaccctgagtccaccactgagacttttgcggcttgtaccttagagatcacgtctcgtcgctgggctggtgtgccgttctacctgcgcaccggtaagcgtcttggtcgccgtgttactgagattgccgtggtgtttaaagacgcaccacaccagcctttcgacggcgacatgactgtatcccttggccaaaacgccatcgtgattcgcgtgcagcctgatgaaggtgtgctcatccgcttcggttccaaggttccaggttctgccatggaagtccgtgacgtcaacatggacttctcctactcagaatccttcactgaagaatcacctgaagcatacgagcgcctcattttggatgcgctgttggatgaatccagcctcttccccaccaacgaggaagtggaactgagctggaagattctggatccaattcttgaagcatgggacgccgatggagaaccagaggattacccagcaggtacgtggggtccaaagagcgctgatgaaatgctttcccgcaacggtcacacctggcgcaggccataa

SEQ ID NO: 5 - protein, 304 aa, Artificial Sequence
  cscK(E.coli)
MSAKVWVLGDAVVDLLPESDGRLLPCPGGAPANVAVGIARLGGTSGFIGRVGDDPFGALMQRTLLTEGVDITYLKQDECHRTSTVLVDLNDQGERSFTFMVRPSADLFLETTDLPCWRHGEWLHLCSIALSAEPSRTSAFTAMTAIRHAGGFVSFDPNIREDLWQDEHLLRLCLRQALQLADVVKLSEEEWRLISGKTQNDQDICALAKEYEIAMLLVTKGAEGVVVCYRGQVHHFAGMSVNCVDSTGAGDAFVAGLLTGLSSTGLSTDEREMRRIIDLAQRCGALAVTAKGAMTALPCRQELE

SEQ ID NO: 6 - DNA, 915 bp, Artificial Sequence
  cscK(E.coli)
atgtcagccaaagtatgggttttaggggatgcggtcgtagatctcttgccagaatcagacgggcgcctactgccttgtcctggcggcgcgccagctaacgttgcggtgggaatcgccagattaggcggaacaagtgggtttataggtcgggtgggggatgatccttttggtgcgttaatgcaaagaacgctgctaactgagggagtcgatatcacgtatctgaagcaagatgaatgtcaccggacatccacggtgcttgtcgatctgaacgatcaaggggaacgttcatttacgtttatggtccgccccagtgccgatctttttttagagacgacagacttgccctgctggcgacatggcgaatggttacatctctgttcaattgcgttgtctgccgagccttcgcgtaccagcgcatttactgcgatgacggcgatccggcatgccggaggttttgtcagcttcgatcctaatattcgtgaagatctatggcaagacgagcatttgctccgcttgtgtttgcggcaggcgctacaactggcggatgtcgtcaagctctcggaagaagaatggcgacttatcagtggaaaaacacagaacgatcaggatatatgcgccctggcaaaagagtatgagatcgccatgctgttggtgactaaaggtgcagaaggggtggtggtctgttatcgaggacaagttcaccattttgctggaatgtctgtgaattgtgtcgatagcacgggggcgggagatgcgttcgttgccgggttactcacaggtctgtcctctacgggattatctacagatgagagagaaatgcgacgaattatcgatctcgctcaacgttgcggagcgcttgcagtaacggcgaaaggggcaatgacagcgctgccatgtcgacaagaactggaatag

SEQ ID NO: 7 - DNA, 40 bp, Artificial Sequence
  primer 1
gcagaaggaatgagttcctcggcgcttcatgtcaacaatc

SEQ ID NO: 8 - DNA, 23 bp, Artificial Sequence
  primer 2
tgttttgatctcctccaataatc

SEQ ID NO: 9 - DNA, 35 bp, Artificial Sequence
  primer 3
tattggaggagatcaaaacagtgagcacaaacacg

SEQ ID NO: 10 - DNA, 40 bp, Artificial Sequence
  primer 4
gttattagatgtcgggcccattatggcctgcgccaggtgt

SEQ ID NO: 11 - DNA, 40 bp, Artificial Sequence
  primer 5
gcagaaggaatgagttcctcagaaacatcccagcgctact

SEQ ID NO: 12 - DNA, 23 bp, Artificial Sequence
  primer 6
gagtgtttcctttcgttgggtac

SEQ ID NO: 13 - DNA, 35 bp, Artificial Sequence
  primer 7
cccaacgaaaggaaacactcgtgagcacaaacacg

SEQ ID NO: 14 - DNA, 40 bp, Artificial Sequence; identical to SEQ ID NO: 10
  primer 8

SEQ ID NO: 15 - DNA, 40 bp, Artificial Sequence; identical to SEQ ID NO: 7
  primer 9

SEQ ID NO: 16 - DNA, 23 bp, Artificial Sequence
  primer 10
tgttttgatctcctccaataatc

SEQ ID NO: 17 - DNA, 35 bp, Artificial Sequence; identical to SEQ ID NO: 9
  primer 11

SEQ ID NO: 18 - DNA, 40 bp, Artificial Sequence; identical to SEQ ID NO: 10
  primer 12

SEQ ID NO: 19 - DNA, 40 bp, Artificial Sequence; identical to SEQ ID NO: 11
  primer 13

SEQ ID NO: 20 - DNA, 23 bp, Artificial Sequence
  primer 14
gagtgtttcctttcgttgggtac

SEQ ID NO: 21 - DNA, 35 bp, Artificial Sequence; identical to SEQ ID NO: 13
  primer 15

SEQ ID NO: 22 - DNA, 40 bp, Artificial Sequence; identical to SEQ ID NO: 10
  primer 16

SEQ ID NO: 23 - DNA, 40 bp, Artificial Sequence; identical to SEQ ID NO: 7
  primer 17

SEQ ID NO: 24 - DNA, 23 bp, Artificial Sequence
  primer 18
tgttttgatctcctccaataatc

SEQ ID NO: 25 - DNA, 35 bp, Artificial Sequence
  primer 19
tattggaggagatcaaaacaatgtcagccaaagta

SEQ ID NO: 26 - DNA, 40 bp, Artificial Sequence
  primer 20
gttattagatgtcgggcccactattccagttcttgtcgac

SEQ ID NO: 27 - DNA, 40 bp, Artificial Sequence; identical to SEQ ID NO: 11
  primer 21

SEQ ID NO: 28 - DNA, 23 bp, Artificial Sequence
  primer 22
gagtgtttcctttcgttgggtac

SEQ ID NO: 29 - DNA, 40 bp, Artificial Sequence
  primer 23
cccaacgaaaggaaacactcatgtcagccaaagtatgggt

SEQ ID NO: 30 - DNA, 40 bp, Artificial Sequence; identical to SEQ ID NO: 26
  primer 24

SEQ ID NO: 31 - DNA, 40 bp, Artificial Sequence; identical to SEQ ID NO: 7
  primer 25

SEQ ID NO: 32 - DNA, 25 bp, Artificial Sequence
  primer 26
ggatgtttctttatggcctgcgcca

SEQ ID NO: 33 - DNA, 25 bp, Artificial Sequence
  primer 27
caggccataaagaaacatcccagcg

SEQ ID NO: 34 - DNA, 40 bp, Artificial Sequence; identical to SEQ ID NO: 26
  primer 28

SEQ ID NO: 35 - DNA, 40 bp, Artificial Sequence; identical to SEQ ID NO: 11
  primer 29

SEQ ID NO: 36 - DNA, 25 bp, Artificial Sequence
  primer 30
atgaagcgccttatggcctgcgcca

SEQ ID NO: 37 - DNA, 25 bp, Artificial Sequence
  primer 31
caggccataaggcgcttcatgtcaa

SEQ ID NO: 38 - DNA, 40 bp, Artificial Sequence; identical to SEQ ID NO: 26
  primer 32

SEQ ID NO: 39 - DNA, 40 bp, Artificial Sequence; identical to SEQ ID NO: 7
  primer 33

SEQ ID NO: 40 - DNA, 25 bp, Artificial Sequence
  primer 34
ggatgtttctttatggcctgcgcca

SEQ ID NO: 41 - DNA, 25 bp, Artificial Sequence
  primer 35
caggccataaagaaacatcccagcg

SEQ ID NO: 42 - DNA, 40 bp, Artificial Sequence; identical to SEQ ID NO: 26
  primer 36

SEQ ID NO: 43 - DNA, 40 bp, Artificial Sequence; identical to SEQ ID NO: 11
  primer 37

SEQ ID NO: 44 - DNA, 25 bp, Artificial Sequence
  primer 38
atgaagcgccttatggcctgcgcca

SEQ ID NO: 45 - DNA, 25 bp, Artificial Sequence
  primer 39
caggccataaggcgcttcatgtcaa

SEQ ID NO: 46 - DNA, 40 bp, Artificial Sequence; identical to SEQ ID NO: 26
  primer 40

SEQ ID NO: 47 - DNA, 20 bp, Artificial Sequence
  primer 41
acgacgctggtatttctccc

SEQ ID NO: 48 - DNA, 20 bp, Artificial Sequence
  primer 42
tgattgtcgatatgaccggg